European Patent Specification EP 3 877 520 B1, published March 19, 2025. Title: WHOLE TRANSCRIPTOME ANALYSIS OF SINGLE CELLS USING RANDOM PRIMING. Applicant: Cellular Research, Inc. Shum, Eleen. The sequence listing filed with the application follows.

SEQUENCE LISTING (9 sequences)

SEQ ID NO: 1 - DNA, 32 bp, Artificial Sequence
  Synthetic Oligonucleotide
  misc_feature (24)..(32): n is a, c, g, or t
tcagacgtgtgctcttccgatctnnnnnnnnn

SEQ ID NO: 2 - DNA, 95 bp, Artificial Sequence
  Synthetic Oligonucleotide
  5'AmMC6 (1)..(1): 5' Amino Modifier C6
gttgtcaagatgctaccgttcagagtacgtggagttggtggcccgaccccgagcgctacgagccccccggaaaaaaaaaaaaaaaaaaaaaaaaa

SEQ ID NO: 3 - DNA, 200 bp, Artificial Sequence
  Synthetic Oligonucleotide
  5AmMC6 (1)..(1): 5' Amino Modifier C6
gttgtcaagatgctaccgttcagagctactgtccgaagttaccgtgtatctaccacgggtggtttttcgaatccggaaaagatagtaataagtgttttagttggaataagtcgcaacttttggagacggttacctctcaatttttctgatccgtaggccccccgatctcggcctcaaaaaaaaaaaaaaaaaaaaaaaaa

SEQ ID NO: 4 - DNA, 25 bp, Artificial Sequence
  Synthetic Oligonucleotide
gttgtcaagatgctaccgttcagag

SEQ ID NO: 5 - DNA, 20 bp, Artificial Sequence
  Synthetic Oligonucleotide
acacgacgctcttccgatct

SEQ ID NO: 6 - DNA, 95 bp, Artificial Sequence
  Synthetic Oligonucleotide
gttgtcaagatgctaccgttcagagccccatgtctagtacctattggtcccctatcctcagattcgtttaaaaaaaaaaaaaaaaaaaaaaaaaa

SEQ ID NO: 7 - DNA, 26 bp, Artificial Sequence
  Synthetic Oligonucleotide
tttttttttttttttttttttttttt

SEQ ID NO: 8 - DNA, 20 bp, Artificial Sequence
  Synthetic Oligonucleotide
aaaaaaaaaaaaaaaaaaaa

SEQ ID NO: 9 - DNA, 20 bp, Artificial Sequence
  Synthetic Oligonucleotide
tttttttttttttttttttt